European Patent Application EP 4 491 708 A1, published January 15, 2025. Title: Microorganism comprising Geranylgeranyl pyrophosphate synthase derived from Haematococcus pluvialis, for producing carotenoid or compound in which a precursor thereof is carotenoid, and method using the same. Applicant: 씨제이제일제당 주식회사. The sequence listing filed with the application follows.

SEQUENCE LISTING (103 sequences)

SEQ ID NO: 1 - DNA, 1017 bp, synthetic construct
  source 1..1017: mol_type = other DNA
atgatccgagccatgcacaaccgagcccccaccccccgaacccgagtgtctcacccccgatctcaccgagccctggcccacgtgtctgccgtggccaccgccggccaggtggccgaggtgcactctgcccccgccttcgacttcgagatgtacatgcgagaccgagccgagatggtgaacaaggccctggacgccgccctgccctctcgataccccgaggtgctggtggactctatgcgatactctgtgctggccggcggcaagcgagtgcgacccgccctgaccctggccgcctgtgacctggtgggcggcgacatggccaccgccctgcccaccgcctgtgccatggagatgatccacaccatgtctctgatccacgacgacctgcccgccatggacaacgacgacttccgacgaggccgacccaccaaccacaaggtgtacggcgaggacatcgccatcctggccggcgacgccctgctgtctttcgccttcgagcacatcgcccgagacaccaagggcgtgcccgccgacgccgtgctgaaggtgatcatggagctgggccgagccgtgggcgcccagggcctgtctgccggccaggccgtggacatcaagtctgagggccaggaggtgggcctggaggtgctggagtacatccaccaccacaagaccgccgccctgctggaggccgccgtggtgtgtggcgccctggtgggcggcgccgacaccgccaccgtggagaagctgcgaaagtacgccctgaacatcggcctggccttccaggtgatcgacgacatcctggacgtgacccagaccaccgagaccctgggcaagaccgccgccaaggacctggccgtgaacaagaccacctaccccaagctgctgggcctggaggcctctcgaaaggtggccgacgacctgatccgagaggccatcgcccagctggacgagttcgagcccgcccgaaaggcccccatggtggccctggcccacctgatcggctaccgaaagaactag

SEQ ID NO: 2 - DNA, 531 bp, synthetic construct
  source 1..531: mol_type = other DNA
agagaccgggttggcggcgcatttgtgtcccaaaaaacagccccaattgccccaattgaccccaaattgacccagtagcgggcccaaccccggcgagagcccccttctccccacatatcaaacctcccccggttcccacacttgccgttaagggcgtagggtactgcagtctggaatctacgcttgttcagactttgtactagtttctttgtctggccatccgggtaacccatgccggacgcaaaatagactactgaaaatttttttgctttgtggttgggactttagccaagggtataaaagaccaccgtccccgaattacctttcctcttcttttctctctctccttgtcaactcacacccgaaatcgttaagcatttccttctgagtataagaatcattcaaaatggtgagtttcagaggcagcagcaattgccacgggctttgagcacacggccgggtgtggtcccattcccatcgacacaagacgccacgtcatccgaccagcactttttgcagtactaaccgcag

SEQ ID NO: 3 - DNA, 254 bp, synthetic construct
  source 1..254: mol_type = other DNA
ctcgagtcatgtaattagttatgtcacgcttacattcacgccctccccccacatccgctctaaccgaaaaggaaggagttagacaacctgaagtctaggtccctatttatttttttatagttatgttagtattaagaacgttatttatatttcaaatttttcttttttttctgtacagacgcgtgtacgcatgtaacattatactgaaaaccttgcttgagaaggttttgggacgctcgaaggctttaatttgc

SEQ ID NO: 4 - DNA, 1799 bp, synthetic construct
  source 1..1799: mol_type = other DNA
agagaccgggttggcggcgcatttgtgtcccaaaaaacagccccaattgccccaattgaccccaaattgacccagtagcgggcccaaccccggcgagagcccccttctccccacatatcaaacctcccccggttcccacacttgccgttaagggcgtagggtactgcagtctggaatctacgcttgttcagactttgtactagtttctttgtctggccatccgggtaacccatgccggacgcaaaatagactactgaaaatttttttgctttgtggttgggactttagccaagggtataaaagaccaccgtccccgaattacctttcctcttcttttctctctctccttgtcaactcacacccgaaatcgttaagcatttccttctgagtataagaatcattcaaaatggtgagtttcagaggcagcagcaattgccacgggctttgagcacacggccgggtgtggtcccattcccatcgacacaagacgccacgtcatccgaccagcactttttgcagtactaaccgcagatccgagccatgcacaaccgagcccccaccccccgaacccgagtgtctcacccccgatctcaccgagccctggcccacgtgtctgccgtggccaccgccggccaggtggccgaggtgcactctgcccccgccttcgacttcgagatgtacatgcgagaccgagccgagatggtgaacaaggccctggacgccgccctgccctctcgataccccgaggtgctggtggactctatgcgatactctgtgctggccggcggcaagcgagtgcgacccgccctgaccctggccgcctgtgacctggtgggcggcgacatggccaccgccctgcccaccgcctgtgccatggagatgatccacaccatgtctctgatccacgacgacctgcccgccatggacaacgacgacttccgacgaggccgacccaccaaccacaaggtgtacggcgaggacatcgccatcctggccggcgacgccctgctgtctttcgccttcgagcacatcgcccgagacaccaagggcgtgcccgccgacgccgtgctgaaggtgatcatggagctgggccgagccgtgggcgcccagggcctgtctgccggccaggccgtggacatcaagtctgagggccaggaggtgggcctggaggtgctggagtacatccaccaccacaagaccgccgccctgctggaggccgccgtggtgtgtggcgccctggtgggcggcgccgacaccgccaccgtggagaagctgcgaaagtacgccctgaacatcggcctggccttccaggtgatcgacgacatcctggacgtgacccagaccaccgagaccctgggcaagaccgccgccaaggacctggccgtgaacaagaccacctaccccaagctgctgggcctggaggcctctcgaaaggtggccgacgacctgatccgagaggccatcgcccagctggacgagttcgagcccgcccgaaaggcccccatggtggccctggcccacctgatcggctaccgaaagaactagctcgagtcatgtaattagttatgtcacgcttacattcacgccctccccccacatccgctctaaccgaaaaggaaggagttagacaacctgaagtctaggtccctatttatttttttatagttatgttagtattaagaacgttatttatatttcaaatttttcttttttttctgtacagacgcgtgtacgcatgtaacattatactgaaaaccttgcttgagaaggttttgggacgctcgaaggctttaatttgc

SEQ ID NO: 5 - DNA, 1533 bp, synthetic construct
  source 1..1533: mol_type = other DNA
tgcctcctgtctgactcgtcattgccgcctttggagtacgactccaactatgagtgtgcttggatcactttgacgatacattcttcgttggaggctgtgggtctgacagctgcgttttcggcgcggttggccgacaacaatatcagctgcaacgtcattgctggctttcatcatgatcacatttttgtcggcaaaggcgacgcccagagagccattgacgttctttctaatttggaccgatagccgtatagtccagtctatctataagttcaactaactcgtaactattaccataacatatacttcactgccccagataaggttccgataaaaagttctgcagactaaatttatttcagtctcctcttcaccaccaaaatgccctcctacgaagctcgagctaacgtccacaagtccgcctttgccgctcgagtgctcaagctcgtggcagccaagaaaaccaacctgtgtgcttctctggatgttaccaccaccaaggagctcattgagcttgccgataaggtcggaccttatgtgtgcatgatcaagacccatatcgacatcattgacgacttcacctacgccggcactgtgctccccctcaaggaacttgctcttaagcacggtttcttcctgttcgaggacagaaagttcgcagatattggcaacactgtcaagcaccagtacaagaacggtgtctaccgaatcgccgagtggtccgatatcaccaacgcccacggtgtacccggaaccggaatcattgctggcctgcgagctggtgccgaggaaactgtctctgaacagaagaaggaggacgtctctgactacgagaactcccagtacaaggagttcctggtcccctctcccaacgagaagctggccagaggtctgctcatgctggccgagctgtcttgcaagggctctctggccactggcgagtactccaagcagaccattgagcttgcccgatccgaccccgagtttgtggttggcttcattgcccagaaccgacctaagggcgactctgaggactggcttattctgacccccggggtgggtcttgacgacaagggagacgctctcggacagcagtaccgaactgttgaggatgtcatgtctaccggaacggatatcataattgtcggccgaggtctgtacggccagaaccgagatcctattgaggaggccaagcgataccagaaggctggctgggaggcttaccagaagattaactgttagaggttagactatggatatgtcatttaactgtgtatatagagagcgtgcaagtatggagcgcttgttcagcttgtatgatggtcagacgacctgtctgatcgagtatgtatgatactgcacaacctgtgtatccgcatgatctgtccaatggggcatgttgttgtgtttctcgatacggagatgctgggtacaagtagctaatacgattgaactacttatacttatatgaggcttgaagaaagctgacttgtgtatgacttattctcaactacatccccagtcacaataccacca

SEQ ID NO: 6 - DNA, 1131 bp, synthetic construct
  source 1..1131: mol_type = other DNA
atggattacgcgaacatcctcacagcaattccactcgagtttactcctcaggatgatatcgtgctccttgaaccgtatcactacctaggaaagaaccctggaaaagaaattcgatcacaactcatcgaggctttcaactattggttggatgtcaagaaggaggatctcgaggtcatccagaacgttgttggcatgctacataccgctagcttattaatggacgatgtggaggattcatcggtcctcaggcgtgggtcgcctgtagcccatctaatttacgggattccgcagacaataaacactgcaaactacgtctactttctggcttatcaagagatcttcaagcttcgcccaacaccgatacccatgcctgtaattcctccttcatctgcttcgcttcaatcaaccgtctcctctgcatcctcctcctcctcggcctcgtctgaaaacgggggcacgtcatctcctaattcgcagattccgttctcgaaagatacgtatcttgataaagtgatcacagacgagatgctttccctccatagagggcaaggcctggagctattctggagagatagtctgacgtgtcctagcgaagaggaatatgtgaaaatggttcttggaaagacgggaggtttgttccgtatagcggtcagattgatgatggcaaagtcagaatgtgacatagactttgtccagcttgtcaacttgatctcaatatacttccagatcagggatgactatatgaaccttcagtcttctgagtatgcccatattaagaattttgcagaggacctcacagaaggaaaattcagttttcccactatccactcgattcgtgccaacccctcatcgagactcgtcatcaatacgttgcagaagaaatcgacctctcctgagatccttcaccactgtgtaaactacatgcgcacagaaacccactcattcgaatatactcaggaagtcctcaacaccttgtcaggtgcactcgagagagaactaggaaggcttcaaggagagttcgcagaagctaactcaaagattgatcttggagacgtagagtcggaaggaagaacggggaagaacgtcaaattggaagcgatcctgaaaaagctagccgatatccctctgtga

SEQ ID NO: 7 - DNA, 500 bp, synthetic construct
  source 1..500: mol_type = other DNA
ctatccgaagatcaagagcgaagcaagttgtaagtccaggacatgtttcccgcccacgcgagtgatttataacacctctcttttttgacacccgctcgccttgaaattcatgtcacataaattatagtcaacgacgtttgaataacttgtcttgtagttcgatgatgatcatatgattacattaatagtaattactgtatttgatatatatactaattacaatagtacatattagaacatacaatagttagtgccgtgaagtggcttaaaataccgcgagtcgattacgtaatattatatataatgtcaaagtggggtcccagagccgaagaaggtgcttttcttgaagatcccagtgtattggacaagtatatctgtctctatgattgtttttccaggtgaaaatgttgaacaaagtgtctactggagtttgtaagcgctggtgcgactggggccacttttaaaacccgccttagcaggctttttcaccgttccaagac

SEQ ID NO: 8 - DNA, 2159 bp, synthetic construct
  source 1..2159: mol_type = other DNA
agagaccgggttggcggcgcatttgtgtcccaaaaaacagccccaattgccccaattgaccccaaattgacccagtagcgggcccaaccccggcgagagcccccttctccccacatatcaaacctcccccggttcccacacttgccgttaagggcgtagggtactgcagtctggaatctacgcttgttcagactttgtactagtttctttgtctggccatccgggtaacccatgccggacgcaaaatagactactgaaaatttttttgctttgtggttgggactttagccaagggtataaaagaccaccgtccccgaattacctttcctcttcttttctctctctccttgtcaactcacacccgaaatcgttaagcatttccttctgagtataagaatcattcaaaatggtgagtttcagaggcagcagcaattgccacgggctttgagcacacggccgggtgtggtcccattcccatcgacacaagacgccacgtcatccgaccagcactttttgcagtactaaccgcaggattacgcgaacatcctcacagcaattccactcgagtttactcctcaggatgatatcgtgctccttgaaccgtatcactacctaggaaagaaccctggaaaagaaattcgatcacaactcatcgaggctttcaactattggttggatgtcaagaaggaggatctcgaggtcatccagaacgttgttggcatgctacataccgctagcttattaatggacgatgtggaggattcatcggtcctcaggcgtgggtcgcctgtagcccatctaatttacgggattccgcagacaataaacactgcaaactacgtctactttctggcttatcaagagatcttcaagcttcgcccaacaccgatacccatgcctgtaattcctccttcatctgcttcgcttcaatcaaccgtctcctctgcatcctcctcctcctcggcctcgtctgaaaacgggggcacgtcatctcctaattcgcagattccgttctcgaaagatacgtatcttgataaagtgatcacagacgagatgctttccctccatagagggcaaggcctggagctattctggagagatagtctgacgtgtcctagcgaagaggaatatgtgaaaatggttcttggaaagacgggaggtttgttccgtatagcggtcagattgatgatggcaaagtcagaatgtgacatagactttgtccagcttgtcaacttgatctcaatatacttccagatcagggatgactatatgaaccttcagtcttctgagtatgcccatattaagaattttgcagaggacctcacagaaggaaaattcagttttcccactatccactcgattcgtgccaacccctcatcgagactcgtcatcaatacgttgcagaagaaatcgacctctcctgagatccttcaccactgtgtaaactacatgcgcacagaaacccactcattcgaatatactcaggaagtcctcaacaccttgtcaggtgcactcgagagagaactaggaaggcttcaaggagagttcgcagaagctaactcaaagattgatcttggagacgtagagtcggaaggaagaacggggaagaacgtcaaattggaagcgatcctgaaaaagctagccgatatccctctgtgactatccgaagatcaagagcgaagcaagttgtaagtccaggacatgtttcccgcccacgcgagtgatttataacacctctcttttttgacacccgctcgccttgaaattcatgtcacataaattatagtcaacgacgtttgaataacttgtcttgtagttcgatgatgatcatatgattacattaatagtaattactgtatttgatatatatactaattacaatagtacatattagaacatacaatagttagtgccgtgaagtggcttaaaataccgcgagtcgattacgtaatattatatataatgtcaaagtggggtcccagagccgaagaaggtgcttttcttgaagatcccagtgtattggacaagtatatctgtctctatgattgtttttccaggtgaaaatgttgaacaaagtgtctactggagtttgtaagcgctggtgcgactggggccacttttaaaacccgccttagcaggctttttcaccgttccaagac

SEQ ID NO: 9 - DNA, 1008 bp, Saccharomyces cerevisiae
  source 1..1008: mol_type = genomic DNA
atggaggccaagatagatgagctgatcaataatgatcctgtttggtccagccaaaatgaaagcttgatttcaaaaccttataatcacatccttttgaaacctggcaagaactttagactaaatttaatagttcaaattaacagagttatgaatttgcccaaagaccagctggccatagtttcgcaaattgttgagctcttgcataattccagccttttaatcgacgatatagaagataatgctcccttgagaaggggacagaccacttctcacttaatcttcggtgtaccctccactataaacaccgcaaattatatgtatttcagagccatgcaacttgtatcgcagctaaccacaaaagagcctttgtatcataatttgattacgattttcaacgaagaattgatcaatctacataggggacaaggcttggatatatactggagagactttctgcctgaaatcatacctactcaggagatgtatttgaatatggttatgaataaaacaggcggccttttcagattaacgttgagactcatggaagcgctgtctccttcctcacaccacggccattcgttggttcctttcataaatcttctgggtattatttatcagattagagatgattacttgaatttgaaagatttccaaatgtccagcgaaaaaggctttgctgaggacattacagaggggaagttatcttttcccatcgtccacgcccttaacttcactaaaacgaaaggtcaaactgagcaacacaatgaaattctaagaattctcctgttgaggacaagtgataaagatataaaactaaagctgattcaaatactggaattcgacaccaattcattggcctacaccaaaaattttattaatcaattagtgaatatgataaaaaatgataatgaaaataagtatttacctgatttggcttcgcattccgacaccgccaccaatttacatgacgaattgttatatataatagaccacttatccgaattgtga

SEQ ID NO: 10 - DNA, 2036 bp, synthetic construct
  source 1..2036: mol_type = other DNA
agagaccgggttggcggcgcatttgtgtcccaaaaaacagccccaattgccccaattgaccccaaattgacccagtagcgggcccaaccccggcgagagcccccttctccccacatatcaaacctcccccggttcccacacttgccgttaagggcgtagggtactgcagtctggaatctacgcttgttcagactttgtactagtttctttgtctggccatccgggtaacccatgccggacgcaaaatagactactgaaaatttttttgctttgtggttgggactttagccaagggtataaaagaccaccgtccccgaattacctttcctcttcttttctctctctccttgtcaactcacacccgaaatcgttaagcatttccttctgagtataagaatcattcaaaatggtgagtttcagaggcagcagcaattgccacgggctttgagcacacggccgggtgtggtcccattcccatcgacacaagacgccacgtcatccgaccagcactttttgcagtactaaccgcaggaggccaagatagatgagctgatcaataatgatcctgtttggtccagccaaaatgaaagcttgatttcaaaaccttataatcacatccttttgaaacctggcaagaactttagactaaatttaatagttcaaattaacagagttatgaatttgcccaaagaccagctggccatagtttcgcaaattgttgagctcttgcataattccagccttttaatcgacgatatagaagataatgctcccttgagaaggggacagaccacttctcacttaatcttcggtgtaccctccactataaacaccgcaaattatatgtatttcagagccatgcaacttgtatcgcagctaaccacaaaagagcctttgtatcataatttgattacgattttcaacgaagaattgatcaatctacataggggacaaggcttggatatatactggagagactttctgcctgaaatcatacctactcaggagatgtatttgaatatggttatgaataaaacaggcggccttttcagattaacgttgagactcatggaagcgctgtctccttcctcacaccacggccattcgttggttcctttcataaatcttctgggtattatttatcagattagagatgattacttgaatttgaaagatttccaaatgtccagcgaaaaaggctttgctgaggacattacagaggggaagttatcttttcccatcgtccacgcccttaacttcactaaaacgaaaggtcaaactgagcaacacaatgaaattctaagaattctcctgttgaggacaagtgataaagatataaaactaaagctgattcaaatactggaattcgacaccaattcattggcctacaccaaaaattttattaatcaattagtgaatatgataaaaaatgataatgaaaataagtatttacctgatttggcttcgcattccgacaccgccaccaatttacatgacgaattgttatatataatagaccacttatccgaattgtgactatccgaagatcaagagcgaagcaagttgtaagtccaggacatgtttcccgcccacgcgagtgatttataacacctctcttttttgacacccgctcgccttgaaattcatgtcacataaattatagtcaacgacgtttgaataacttgtcttgtagttcgatgatgatcatatgattacattaatagtaattactgtatttgatatatatactaattacaatagtacatattagaacatacaatagttagtgccgtgaagtggcttaaaataccgcgagtcgattacgtaatattatatataatgtcaaagtggggtcccagagccgaagaaggtgcttttcttgaagatcccagtgtattggacaagtatatctgtctctatgattgtttttccaggtgaaaatgttgaacaaagtgtctactggagtttgtaagcgctggtgcgactggggccacttttaaaacccgccttagcaggctttttcaccgttccaagac

SEQ ID NO: 11 - DNA, 984 bp, Yarrowia lipolytica
  source 1..984: mol_type = genomic DNA
atggattataacagcgcggatttcaaggagatatggggcaaggccgccgacaccgcgctgctgggaccgtacaactacctcgccaacaaccggggccacaacatcagagaacacttgatcgcagcgttcggagcggttatcaaggtggacaagagcgatctcgagaccatttcgcacatcaccaagattttgcataactcgtcgctgcttgttgatgacgtggaagacaactcgatgctccgacgaggcctgccggcagcccattgtctgtttggagtcccccaaaccatcaactccgccaactacatgtactttgtggctctgcaggaggtgctcaagctcaagtcttatgatgccgtctccattttcaccgaggaaatgatcaacttgcatagaggtcagggtatggatctctactggagagaaacactcacttgcccctcggaagacgagtatctggagatggtggtgcacaagaccggtggactgtttcggctggctctgagacttatgctgtcggtggcatcgaaacaggaggaccatgaaaagatcaactttgatctcacacaccttaccgacacactgggagtcatttaccagattctggatgattacctcaacctgcagtccacggaattgaccgagaacaagggattctgcgaagatatcagcgaaggaaagttttcgtttccgctgattcacagcatacgcaccaacccggataaccacgagattctcaacattctcaaacagcgaacaagcgacgcttcactcaaaaagtacgccgtggactacatgagaacagaaaccaagagtttcgactactgcctcaagaggatacaggccatgtcactcaaggcaagttcgtacattgatgatctagcagcagctggccacgatgtctccaagctacgagccattttgcattattttgtgtccacctctgactgtgaggagagaaagtactttgaggatgcgcagtga

SEQ ID NO: 12 - DNA, 2012 bp, synthetic construct
  source 1..2012: mol_type = other DNA
agagaccgggttggcggcgcatttgtgtcccaaaaaacagccccaattgccccaattgaccccaaattgacccagtagcgggcccaaccccggcgagagcccccttctccccacatatcaaacctcccccggttcccacacttgccgttaagggcgtagggtactgcagtctggaatctacgcttgttcagactttgtactagtttctttgtctggccatccgggtaacccatgccggacgcaaaatagactactgaaaatttttttgctttgtggttgggactttagccaagggtataaaagaccaccgtccccgaattacctttcctcttcttttctctctctccttgtcaactcacacccgaaatcgttaagcatttccttctgagtataagaatcattcaaaatggtgagtttcagaggcagcagcaattgccacgggctttgagcacacggccgggtgtggtcccattcccatcgacacaagacgccacgtcatccgaccagcactttttgcagtactaaccgcaggattataacagcgcggatttcaaggagatatggggcaaggccgccgacaccgcgctgctgggaccgtacaactacctcgccaacaaccggggccacaacatcagagaacacttgatcgcagcgttcggagcggttatcaaggtggacaagagcgatctcgagaccatttcgcacatcaccaagattttgcataactcgtcgctgcttgttgatgacgtggaagacaactcgatgctccgacgaggcctgccggcagcccattgtctgtttggagtcccccaaaccatcaactccgccaactacatgtactttgtggctctgcaggaggtgctcaagctcaagtcttatgatgccgtctccattttcaccgaggaaatgatcaacttgcatagaggtcagggtatggatctctactggagagaaacactcacttgcccctcggaagacgagtatctggagatggtggtgcacaagaccggtggactgtttcggctggctctgagacttatgctgtcggtggcatcgaaacaggaggaccatgaaaagatcaactttgatctcacacaccttaccgacacactgggagtcatttaccagattctggatgattacctcaacctgcagtccacggaattgaccgagaacaagggattctgcgaagatatcagcgaaggaaagttttcgtttccgctgattcacagcatacgcaccaacccggataaccacgagattctcaacattctcaaacagcgaacaagcgacgcttcactcaaaaagtacgccgtggactacatgagaacagaaaccaagagtttcgactactgcctcaagaggatacaggccatgtcactcaaggcaagttcgtacattgatgatctagcagcagctggccacgatgtctccaagctacgagccattttgcattattttgtgtccacctctgactgtgaggagagaaagtactttgaggatgcgcagtgactatccgaagatcaagagcgaagcaagttgtaagtccaggacatgtttcccgcccacgcgagtgatttataacacctctcttttttgacacccgctcgccttgaaattcatgtcacataaattatagtcaacgacgtttgaataacttgtcttgtagttcgatgatgatcatatgattacattaatagtaattactgtatttgatatatatactaattacaatagtacatattagaacatacaatagttagtgccgtgaagtggcttaaaataccgcgagtcgattacgtaatattatatataatgtcaaagtggggtcccagagccgaagaaggtgcttttcttgaagatcccagtgtattggacaagtatatctgtctctatgattgtttttccaggtgaaaatgttgaacaaagtgtctactggagtttgtaagcgctggtgcgactggggccacttttaaaacccgccttagcaggctttttcaccgttccaagac

SEQ ID NO: 13 - DNA, 828 bp, synthetic construct
  source 1..828: mol_type = other DNA
atgggcctgatgctgatcgactggtgtgccctggccctggtggtgttcatcggcctgccccacggcgccctggacgccgccatctctttctctatgatctcttctgccaagcgaatcgcccgactggccggcatcctgctgatctacctgctgctggccaccgccttcttcctgatctggtaccagctgcccgccttctctctgctgatcttcctgctgatctctatcatccacttcggcatggccgacttcaacgcctctccctctaagctgaagtggccccacatcatcgcccacggcggcgtggtgaccgtgtggctgcccctgatccagaagaacgaggtgaccaagctgttctctatcctgaccaacggccccacccccatcctgtgggacatcctgctgatcttcttcctgtgttggtctatcggcgtgtgtctgcacacctacgagaccctgcgatctaagcactacaacatcgccttcgagctgatcggcctgatcttcctggcctggtacgccccccccctggtgaccttcgccacctacttctgtttcatccactctcgacgacacttctctttcgtgtggaagcagctgcagcacatgtcttctaagaagatgatgatcggctctgccatcatcctgtcttgtacctcttggctgatcggcggcggcatctacttcttcctgaactctaagatgatcgcctctgaggccgccctgcagaccgtgttcatcggcctggccgccctgaccgtgccccacatgatcctgatcgacttcatcttccgaccccactcttctcgaatcaagatcaagaactag

SEQ ID NO: 14 - DNA, 1610 bp, synthetic construct
  source 1..1610: mol_type = other DNA
agagaccgggttggcggcgcatttgtgtcccaaaaaacagccccaattgccccaattgaccccaaattgacccagtagcgggcccaaccccggcgagagcccccttctccccacatatcaaacctcccccggttcccacacttgccgttaagggcgtagggtactgcagtctggaatctacgcttgttcagactttgtactagtttctttgtctggccatccgggtaacccatgccggacgcaaaatagactactgaaaatttttttgctttgtggttgggactttagccaagggtataaaagaccaccgtccccgaattacctttcctcttcttttctctctctccttgtcaactcacacccgaaatcgttaagcatttccttctgagtataagaatcattcaaaatggtgagtttcagaggcagcagcaattgccacgggctttgagcacacggccgggtgtggtcccattcccatcgacacaagacgccacgtcatccgaccagcactttttgcagtactaaccgcagggcctgatgctgatcgactggtgtgccctggccctggtggtgttcatcggcctgccccacggcgccctggacgccgccatctctttctctatgatctcttctgccaagcgaatcgcccgactggccggcatcctgctgatctacctgctgctggccaccgccttcttcctgatctggtaccagctgcccgccttctctctgctgatcttcctgctgatctctatcatccacttcggcatggccgacttcaacgcctctccctctaagctgaagtggccccacatcatcgcccacggcggcgtggtgaccgtgtggctgcccctgatccagaagaacgaggtgaccaagctgttctctatcctgaccaacggccccacccccatcctgtgggacatcctgctgatcttcttcctgtgttggtctatcggcgtgtgtctgcacacctacgagaccctgcgatctaagcactacaacatcgccttcgagctgatcggcctgatcttcctggcctggtacgccccccccctggtgaccttcgccacctacttctgtttcatccactctcgacgacacttctctttcgtgtggaagcagctgcagcacatgtcttctaagaagatgatgatcggctctgccatcatcctgtcttgtacctcttggctgatcggcggcggcatctacttcttcctgaactctaagatgatcgcctctgaggccgccctgcagaccgtgttcatcggcctggccgccctgaccgtgccccacatgatcctgatcgacttcatcttccgaccccactcttctcgaatcaagatcaagaactagctcgagtcatgtaattagttatgtcacgcttacattcacgccctccccccacatccgctctaaccgaaaaggaaggagttagacaacctgaagtctaggtccctatttatttttttatagttatgttagtattaagaacgttatttatatttcaaatttttcttttttttctgtacagacgcgtgtacgcatgtaacattatactgaaaaccttgcttgagaaggttttgggacgctcgaaggctttaatttgc

SEQ ID NO: 15 - DNA, 24 bp, synthetic construct
  source 1..24: mol_type = other DNA
catcatttcaaaagagggaacagc

SEQ ID NO: 16 - DNA, 41 bp, synthetic construct
  source 1..41: mol_type = other DNA
cgccgccaacccggtctctgtgtttggcggtgtgagttgtc

SEQ ID NO: 17 - DNA, 41 bp, synthetic construct
  source 1..41: mol_type = other DNA
gacaactcacaccgccaaacacagagaccgggttggcggcg

SEQ ID NO: 18 - DNA, 45 bp, synthetic construct
  source 1..45: mol_type = other DNA
cggttgtgcatggctcggatctgcggttagtactgcaaaaagtgc

SEQ ID NO: 19 - DNA, 45 bp, synthetic construct
  source 1..45: mol_type = other DNA
gcactttttgcagtactaaccgcagatccgagccatgcacaaccg

SEQ ID NO: 20 - DNA, 40 bp, synthetic construct
  source 1..40: mol_type = other DNA
aactaattacatgactcgagctagttctttcggtagccga

SEQ ID NO: 21 - DNA, 40 bp, synthetic construct
  source 1..40: mol_type = other DNA
tcggctaccgaaagaactagctcgagtcatgtaattagtt

SEQ ID NO: 22 - DNA, 40 bp, synthetic construct
  source 1..40: mol_type = other DNA
gacgagtcagacaggaggcagcaaattaaagccttcgagc

SEQ ID NO: 23 - DNA, 40 bp, synthetic construct
  source 1..40: mol_type = other DNA
gctcgaaggctttaatttgctgcctcctgtctgactcgtc

SEQ ID NO: 24 - DNA, 40 bp, synthetic construct
  source 1..40: mol_type = other DNA
aactaattacatgactcgagtggtggtattgtgactgggg

SEQ ID NO: 25 - DNA, 40 bp, synthetic construct
  source 1..40: mol_type = other DNA
ccccagtcacaataccaccactcgagtcatgtaattagtt

SEQ ID NO: 26 - DNA, 44 bp, synthetic construct
  source 1..44: mol_type = other DNA
ccatatggagtgttatttgaaggggcaaattaaagccttcgagc

SEQ ID NO: 27 - DNA, 44 bp, synthetic construct
  source 1..44: mol_type = other DNA
gctcgaaggctttaatttgccccttcaaataacactccatatgg

SEQ ID NO: 28 - DNA, 21 bp, synthetic construct
  source 1..21: mol_type = other DNA
ccgatacagtgtccaagtacg

SEQ ID NO: 29 - DNA, 22 bp, synthetic construct
  source 1..22: mol_type = other DNA
gagtgtctgaagacaaggcttc

SEQ ID NO: 30 - DNA, 20 bp, synthetic construct
  source 1..20: mol_type = other DNA
gacgacaatgctgagctccg

SEQ ID NO: 31 - DNA, 24 bp, synthetic construct
  source 1..24: mol_type = other DNA
catcatttcaaaagagggaacagc

SEQ ID NO: 32 - DNA, 41 bp, synthetic construct; identical to SEQ ID NO: 16
  source 1..41: mol_type = other DNA

SEQ ID NO: 33 - DNA, 41 bp, synthetic construct; identical to SEQ ID NO: 17
  source 1..41: mol_type = other DNA

SEQ ID NO: 34 - DNA, 47 bp, synthetic construct
  source 1..47: mol_type = other DNA
ctgtgaggatgttcgcgtaatcctgcggttagtactgcaaaaagtgc

SEQ ID NO: 35 - DNA, 47 bp, synthetic construct
  source 1..47: mol_type = other DNA
gcactttttgcagtactaaccgcaggattacgcgaacatcctcacag

SEQ ID NO: 36 - DNA, 44 bp, synthetic construct
  source 1..44: mol_type = other DNA
cttcgctcttgatcttcggatagtcacagagggatatcggctag

SEQ ID NO: 37 - DNA, 44 bp, synthetic construct
  source 1..44: mol_type = other DNA
ctagccgatatccctctgtgactatccgaagatcaagagcgaag

SEQ ID NO: 38 - DNA, 45 bp, synthetic construct
  source 1..45: mol_type = other DNA
gacgagtcagacaggaggcagtcttggaacggtgaaaaagcctgc

SEQ ID NO: 39 - DNA, 45 bp, synthetic construct
  source 1..45: mol_type = other DNA
gcaggctttttcaccgttccaagactgcctcctgtctgactcgtc

SEQ ID NO: 40 - DNA, 41 bp, synthetic construct
  source 1..41: mol_type = other DNA
cgctcttgatcttcggatagtggtggtattgtgactgggga

SEQ ID NO: 41 - DNA, 41 bp, synthetic construct
  source 1..41: mol_type = other DNA
tccccagtcacaataccaccactatccgaagatcaagagcg

SEQ ID NO: 42 - DNA, 48 bp, synthetic construct
  source 1..48: mol_type = other DNA
catatggagtgttatttgaaggggtcttggaacggtgaaaaagcctgc

SEQ ID NO: 43 - DNA, 48 bp, synthetic construct
  source 1..48: mol_type = other DNA
gcaggctttttcaccgttccaagaccccttcaaataacactccatatg

SEQ ID NO: 44 - DNA, 21 bp, synthetic construct
  source 1..21: mol_type = other DNA
ccgatacagtgtccaagtacg

SEQ ID NO: 45 - DNA, 22 bp, synthetic construct
  source 1..22: mol_type = other DNA
gagtgtctgaagacaaggcttc

SEQ ID NO: 46 - DNA, 20 bp, synthetic construct
  source 1..20: mol_type = other DNA
gacgacaatgctgagctccg

SEQ ID NO: 47 - DNA, 46 bp, synthetic construct
  source 1..46: mol_type = other DNA
cagctcatctatcttggcctcctgcggttagtactgcaaaaagtgc

SEQ ID NO: 48 - DNA, 46 bp, synthetic construct
  source 1..46: mol_type = other DNA
gcactttttgcagtactaaccgcaggaggccaagatagatgagctg

SEQ ID NO: 49 - DNA, 57 bp, synthetic construct
  source 1..57: mol_type = other DNA
cttcgctcttgatcttcggatagtcacaattcggataagtggtctattatatataac

SEQ ID NO: 50 - DNA, 57 bp, synthetic construct
  source 1..57: mol_type = other DNA
gttatatataatagaccacttatccgaattgtgactatccgaagatcaagagcgaag

SEQ ID NO: 51 - DNA, 49 bp, synthetic construct
  source 1..49: mol_type = other DNA
cttgaaatccgcgctgttataatcctgcggttagtactgcaaaaagtgc

SEQ ID NO: 52 - DNA, 49 bp, synthetic construct
  source 1..49: mol_type = other DNA
gcactttttgcagtactaaccgcaggattataacagcgcggatttcaag

SEQ ID NO: 53 - DNA, 45 bp, synthetic construct
  source 1..45: mol_type = other DNA
cttcgctcttgatcttcggatagtcactgcgcatcctcaaagtac

SEQ ID NO: 54 - DNA, 45 bp, synthetic construct
  source 1..45: mol_type = other DNA
gtactttgaggatgcgcagtgactatccgaagatcaagagcgaag

SEQ ID NO: 55 - DNA, 25 bp, synthetic construct
  source 1..25: mol_type = other DNA
ggcgtttcaggtggttgcgtgagtg

SEQ ID NO: 56 - DNA, 53 bp, synthetic construct
  source 1..53: mol_type = other DNA
gacacaaatgcgccgccaacccggtctctgcggcggttcgtggttcgtgtttc

SEQ ID NO: 57 - DNA, 53 bp, synthetic construct
  source 1..53: mol_type = other DNA
gaaacacgaaccacgaaccgccgcagagaccgggttggcggcgcatttgtgtc

SEQ ID NO: 58 - DNA, 40 bp, synthetic construct
  source 1..40: mol_type = other DNA
cagtcgatcagcatcaggccctgcggttagtactgcaaaa

SEQ ID NO: 59 - skipped

SEQ ID NO: 60 - DNA, 40 bp, synthetic construct
  source 1..40: mol_type = other DNA
aactaattacatgactcgagctagttcttgatcttgattc

SEQ ID NO: 61 - DNA, 40 bp, synthetic construct
  source 1..40: mol_type = other DNA
gaatcaagatcaagaactagctcgagtcatgtaattagtt

SEQ ID NO: 62 - DNA, 45 bp, synthetic construct
  source 1..45: mol_type = other DNA
gacgagtcagacaggaggcagcaaattaaagccttcgagcgtccc

SEQ ID NO: 63 - DNA, 45 bp, synthetic construct
  source 1..45: mol_type = other DNA
gggacgctcgaaggctttaatttgctgcctcctgtctgactcgtc

SEQ ID NO: 64 - DNA, 40 bp, synthetic construct; identical to SEQ ID NO: 24
  source 1..40: mol_type = other DNA

SEQ ID NO: 65 - DNA, 40 bp, synthetic construct; identical to SEQ ID NO: 25
  source 1..40: mol_type = other DNA

SEQ ID NO: 66 - DNA, 48 bp, synthetic construct
  source 1..48: mol_type = other DNA
gcagcagtcatacatgttctgaggcaaattaaagccttcgagcgtccc

SEQ ID NO: 67 - DNA, 48 bp, synthetic construct
  source 1..48: mol_type = other DNA
gggacgctcgaaggctttaatttgcctcagaacatgtatgactgctgc

SEQ ID NO: 68 - DNA, 25 bp, synthetic construct
  source 1..25: mol_type = other DNA
ctactttgtgcagattgaggccaag

SEQ ID NO: 69 - DNA, 20 bp, synthetic construct
  source 1..20: mol_type = other DNA
gtcgtctgtcttctcttcag

SEQ ID NO: 70 - DNA, 20 bp, synthetic construct
  source 1..20: mol_type = other DNA
ccaccaagatgggcaagaag

SEQ ID NO: 71 - DNA, 2022 bp, Xanthophyllomyces dendrorhous
  source 1..2022: mol_type = genomic DNA
atgacggctctcgcatattaccagatccatctgatctatactctcccaattcttggtcttctcggcctgctcacttccccgattttgacaaaatttgacatctacaaaatatcgatcctcgtatttattgcgtttagtgcaaccacaccatgggactcatggatcatcagaaatggcgcatggacatatccatcagcggagagtggccaaggcgtgtttggaacgtttctagatgttccatatgaagagtacgctttctttgtcattcaaaccgtaatcaccggcttggtctacgtcttggcaactaggcaccttctcccatctctcgcgcttcccaagactagatcgtccgccctttctctcgcgctcaaggcgctcatccctctgcccattatctacctatttaccgctcaccccagcccatcgcccgacccgctcgtgacagatcactacttctacatgcgggcactctccttactcatcaccccacctaccatgctcttggcagcattatcaggcgaatatgctttcgattggaaaagtggccgagcaaagtcaactattgcagcaatcatgatcccgacggtgtatctgatttgggtagattatgttgctgtcggtcaagactcttggtcgatcaacgatgagaagattgtagggtggaggcttggaggtgtactacccattgaggaagctatgttcttcttactgacgaatctaatgattgttctgggtctgtctgcctgcgatcatactcaggccctatacctgctacacggtcgaactatttatggcaacaaaaagatgccatcttcatttcccctcattacaccgcctgtgctctccctgttttttagcagccgaccatactcttctcagccaaaacgtgacttggaactggcagtcaagttgttggaggaaaagagccggagcttttttgttgcctcggctggatttcctagcgaagttagggagaggctggttggactatacgcattctgccgggtgactgatgatcttatcgactctcctgaagtatcttccaacccgcatgccacaattgacatggtctccgattttcttaccctactatttgggcccccgctacacccttcgcaacctgacaagatcctttcttcgcctttacttcctccttcgcacccttcccgacccacgggaatgtatcccctcccgcctcctccttcgctctcgcctgccgagctcgttcaattccttaccgaaagggttcccgttcaataccatttcgccttcaggttgctcgctaagttgcaagggctgatccctcgatacccactcgacgaactccttagaggatacaccactgatcttatctttcccttatcgacagaggcagtccaggctcggaagacgcctatcgagaccacagctgacttgctggactatggtctatgtgtagcaggctcagtcgccgagctattggtctatgtctcttgggcaagtgcaccaagtcaggtccctgccaccatagaagaaagagaagctgtgttagtggcaagccgagagatgggaactgcccttcagttggtgaacattgctagggacattaaaggggacgcaacagaagggagattttacctaccactctcattctttggtcttcgggatgaatcaaagcttgcgatcccgactgattggacggaacctcggcctcaagatttcgacaaactcctcagtctatctccttcgtccacattaccatcttcaaacgcctcagaaagcttccggttcgaatggaagacgtactcgcttccattagtcgcctacgcagaggatcttgccaaacattcttataagggaattgaccgacttcctaccgaggttcaagcgggaatgcgagcggcttgcgcgagctacctactgatcggccgagagatcaaagtcgtttggaaaggagacgtcggagagagaaggacagttgccggatggaggagagtacggaaagtcttgagtgtggtcatgagcggatgggaagggcagtaa

SEQ ID NO: 72 - DNA, 1749 bp, Xanthophyllomyces dendrorhous
  source 1..1749: mol_type = genomic DNA
atgggaaaagaacaagatcaggataaacccacagctatcatcgtgggatgtggtatcggtggaatcgccactgccgctcgtcttgctaaagaaggtttccaggtcacggtgttcgagaagaacgactactccggaggtcgatgctctttaatcgagcgagatggttatcgattcgatcaggggcccagtttgctgctcttgccagatctcttcaagcagacattcgaagatttgggagagaagatggaagattgggtcgatctcatcaagtgtgaacccaactatgtttgccacttccacgatgaagagactttcactctttcaaccgacatggcgttgctcaagcgggaagtcgagcgttttgaaggcaaagatggatttgatcggttcttgtcgtttatccaagaagcccacagacattacgagcttgctgtcgttcacgtcctgcagaagaacttccctggcttcgcagcattcttacggctacagttcattggccaaatcctggctcttcaccccttcgagtctatctggacaagagtttgtcgatatttcaagaccgacagattacgaagagtcttctcgtttgcagtgatgtacatgggtcaaagcccatacagtgcgcccggaacatattccttgctccaatacaccgaattgaccgagggcatctggtatccgagaggaggcttttggcaggttcctaatactcttcttcagatcgtcaagcgcaacaatccctcagccaagttcaatttcaacgctccagtttcccaggttcttctctctcctgccaaggaccgagcgactggtgttcgacttgaatccggcgaggaacatcacgccgatgttgtgattgtcaatgctgacctcgtttacgcctccgagcacttgattcctgacgatgccagaaacaagattggccaactgggtgaagtcaagagaagttggtgggctgacttagttggtggaaagaagctcaagggaagttgcagtagtttgagcttctactggagcatggaccgaatcgtggacggtctgggcggacacaatatcttcttggccgaggacttcaagggatcattcgacacaatcttcgaggagttgggtctcccagccgatccttccttttacgtgaacgttccctcgcgaatcgatccttctgccgctcccgaaggcaaagatgctatcgtcattcttgtgccgtgtggccatatcgacgcttcgaaccctcaagattacaacaagcttgttgctcgggcaaggaagtttgtgatccacacgctttccgccaagcttggacttcccgactttgaaaaaatgattgtggcagagaaggttcacgatgctccctcttgggagaaagaattcaacctcaaggacggaagcatcttgggactggctcacaactttatgcaagttcttggtttcaggccgagcaccagacatcccaagtatgacaagttgttctttgtcggggcttcgactcatcccggaactggggttcccatcgtcttggctggagccaagttaactgccaaccaagttctcgaatcctttgaccgatccccagctccagatcccaatatgtcactctccgtaccatatggaaaacctctcaaatcaaatggaacgggtatcgattctcaggtccagctgaagttcatggatttggagagatgggtataccttttggtgttgttgattggggccgtgatcgctcgatccgttggtgttcttgctttctga

SEQ ID NO: 73 - DNA, 2804 bp, synthetic construct
  source 1..2804: mol_type = other DNA
agagaccgggttggcggcgcatttgtgtcccaaaaaacagccccaattgccccaattgaccccaaattgacccagtagcgggcccaaccccggcgagagcccccttctccccacatatcaaacctcccccggttcccacacttgccgttaagggcgtagggtactgcagtctggaatctacgcttgttcagactttgtactagtttctttgtctggccatccgggtaacccatgccggacgcaaaatagactactgaaaatttttttgctttgtggttgggactttagccaagggtataaaagaccaccgtccccgaattacctttcctcttcttttctctctctccttgtcaactcacacccgaaatcgttaagcatttccttctgagtataagaatcattcaaaatggtgagtttcagaggcagcagcaattgccacgggctttgagcacacggccgggtgtggtcccattcccatcgacacaagacgccacgtcatccgaccagcactttttgcagtactaaccgcagacggctctcgcatattaccagatccatctgatctatactctcccaattcttggtcttctcggtctgctcacttccccgattttgacaaaatttgacatctacaaaatatcgatcctcgtatttattgcgtttagtgcaaccacaccatgggactcatggatcatcagaaatggcgcatggacatatccatcagcggagagtggccaaggcgtgtttggaacgtttctagatgttccatatgaagagtacgctttctttgtcattcaaaccgtaatcaccggcttggtctacgtcttggcaactaggcaccttctcccatctctcgcgcttcccaagactagatcgtccgccctttctctcgcgctcaaggcgctcatccctctgcccattatctacctatttaccgctcaccccagcccatcgcccgacccgctcgtgacagatcactacttctacatgcgggcactctccttactcatcaccccacctaccatgctcttggcagcattatcaggcgaatatgctttcgattggaaaagtggccgagcaaagtcaactattgcagcaatcatgatcccgacggtgtatctgatttgggtagattatgttgctgtcggtcaagactcttggtcgatcaacgatgagaagattgtagggtggaggcttggaggtgtactacccattgaggaagctatgttcttcttactgacgaatctaatgattgttctgggtctgtctgcctgcgatcatactcaggccctatacctgctacacggtcgaactatttatggcaacaaaaagatgccatcttcatttcccctcattacaccgcctgtgctctccctgttttttagcagccgaccatactcttctcagccaaaacgtgacttggaactggcagtcaagttgttggaggaaaagagccggagcttttttgttgcctcggctggatttcctagcgaagttagggagaggctggttggactatacgcattctgccgggtgactgatgatcttatcgactctcctgaagtatcttccaacccgcatgccacaattgacatggtctccgattttcttaccctactatttgggcccccgctacacccttcgcaacctgacaagatcctttcttcgcctttacttcctccttcgcacccttcccgacccacgggaatgtatcccctcccgcctcctccttcgctctcgcctgccgagctcgttcaattccttaccgaaagggttcccgttcaataccatttcgccttcaggttgctcgctaagttgcaagggctgatccctcgatacccactcgacgaactccttagaggatacaccactgatcttatctttcctttatcgacagaggcagtccaggctcggaagacgcctatcgagaccacagctgacttgctggactatggtctatgtgtagcaggctcagtcgccgagctattggtctatgtctcttgggcaagtgcaccaagtcaggtccctgccaccatagaagaaagagaagctgtgttagtggcaagccgagagatgggaactgcccttcagttggtgaacattgctagggacattaaaggggacgcaacagaagggagattttacctaccactctcattctttggtcttcgggatgaatcaaagcttgcgatcccgactgattggacggaacctcggcctcaagatttcgacaaactcctcagtctatctccttcgtccacattaccatcttcaaacgcctcagaaagcttccggttcgaatggaagacgtactcgcttccattagtcgcctacgcagaggatcttgccaaacattcttataagggaattgaccgacttcctaccgaggttcaagcgggaatgcgagcggcttgcgcgagctacctactgatcggccgagagatcaaagtcgtttggaaaggagacgtcggagagagaaggacagttgccggatggaggagagtacggaaagtcttgagtgtggtcatgagcggatgggaagggcagtaactcgagtcatgtaattagttatgtcacgcttacattcacgccctccccccacatccgctctaaccgaaaaggaaggagttagacaacctgaagtctaggtccctatttatttttttatagttatgttagtattaagaacgttatttatatttcaaatttttcttttttttctgtacagacgcgtgtacgcatgtaacattatactgaaaaccttgcttgagaaggttttgggacgctcgaaggctttaatttgc

SEQ ID NO: 74 - DNA, 2531 bp, synthetic construct
  source 1..2531: mol_type = other DNA
agagaccgggttggcggcgcatttgtgtcccaaaaaacagccccaattgccccaattgaccccaaattgacccagtagcgggcccaaccccggcgagagcccccttctccccacatatcaaacctcccccggttcccacacttgccgttaagggcgtagggtactgcagtctggaatctacgcttgttcagactttgtactagtttctttgtctggccatccgggtaacccatgccggacgcaaaatagactactgaaaatttttttgctttgtggttgggactttagccaagggtataaaagaccaccgtccccgaattacctttcctcttcttttctctctctccttgtcaactcacacccgaaatcgttaagcatttccttctgagtataagaatcattcaaaatggtgagtttcagaggcagcagcaattgccacgggctttgagcacacggccgggtgtggtcccattcccatcgacacaagacgccacgtcatccgaccagcactttttgcagtactaaccgcagggaaaagaacaagatcaggataaacccacagctatcatcgtgggatgtggtatcggtggaatcgccactgccgctcgtcttgctaaagaaggtttccaggtcacggtgttcgagaagaacgactactccggaggtcgatgctctttaatcgagcgagatggttatcgattcgatcaggggcccagtttgctgctcttgccagatctcttcaagcagacattcgaagatttgggagagaagatggaagattgggtcgatctcatcaagtgtgaacccaactatgtttgccacttccacgatgaagagactttcactctttcaaccgacatggcgttgctcaagcgggaagtcgagcgttttgaaggcaaagatggatttgatcggttcttgtcgtttatccaagaagcccacagacattacgagcttgctgtcgttcacgtcctgcagaagaacttccctggcttcgcagcattcttacggctacagttcattggccaaatcctggctcttcaccccttcgagtctatctggacaagagtttgtcgatatttcaagaccgacagattacgaagagtcttctcgtttgcagtgatgtacatgggtcaaagcccatacagtgcgcccggaacatattccttgctccaatacaccgaattgaccgagggcatctggtatccgagaggaggcttttggcaggttcctaatactcttcttcagatcgtcaagcgcaacaatccctcagccaagttcaatttcaacgctccagtttcccaggttcttctctctcctgccaaggaccgagcgactggtgttcgacttgaatccggcgaggaacatcacgccgatgttgtgattgtcaatgctgacctcgtttacgcctccgagcacttgattcctgacgatgccagaaacaagattggccaactgggtgaagtcaagagaagttggtgggctgacttagttggtggaaagaagctcaagggaagttgcagtagtttgagcttctactggagcatggaccgaatcgtggacggtctgggcggacacaatatcttcttggccgaggacttcaagggatcattcgacacaatcttcgaggagttgggtctcccagccgatccttccttttacgtgaacgttccctcgcgaatcgatccttctgccgctcccgaaggcaaagatgctatcgtcattcttgtgccgtgtggccatatcgacgcttcgaaccctcaagattacaacaagcttgttgctcgggcaaggaagtttgtgatccacacgctttccgccaagcttggacttcccgactttgaaaaaatgattgtggcagagaaggttcacgatgctccctcttgggagaaagaattcaacctcaaggacggaagcatcttgggactggctcacaactttatgcaagttcttggtttcaggccgagcaccagacatcccaagtatgacaagttgttctttgtcggggcttcgactcatcccggaactggggttcccatcgtcttggctggagccaagttaactgccaaccaagttctcgaatcctttgaccgatccccagctccagatcccaatatgtcactctccgtaccatatggaaaacctctcaaatcaaatggaacgggtatcgattctcaggtccagctgaagttcatggatttggagagatgggtataccttttggtattgttgattggggccgtgatcgctcgatccgttggtgttcttgctttctgactcgagtcatgtaattagttatgtcacgcttacattcacgccctccccccacatccgctctaaccgaaaaggaaggagttagacaacctgaagtctaggtccctatttatttttttatagttatgttagtattaagaacgttatttatatttcaaatttttcttttttttctgtacagacgcgtgtacgcatgtaacattatactgaaaaccttgcttgagaaggttttgggacgctcgaaggctttaatttgc

SEQ ID NO: 75 - DNA, 1533 bp, Yarrowia lipolytica; identical to SEQ ID NO: 5
  source 1..1533: mol_type = genomic DNA

SEQ ID NO: 76 - DNA, 30 bp, synthetic construct
  source 1..30: mol_type = other DNA
gtgcgcttctctcgtctcggtaaccctgtc

SEQ ID NO: 77 - DNA, 44 bp, synthetic construct
  source 1..44: mol_type = other DNA
atgcgccgccaacccggtctctggggtgtggtggatggggtgtg

SEQ ID NO: 78 - DNA, 44 bp, synthetic construct
  source 1..44: mol_type = other DNA
cacaccccatccaccacaccccagagaccgggttggcggcgcat

SEQ ID NO: 79 - DNA, 39 bp, synthetic construct
  source 1..39: mol_type = other DNA
cgccgccaacccggtctcttgaagacgaaagggcctccg

SEQ ID NO: 80 - DNA, 39 bp, synthetic construct
  source 1..39: mol_type = other DNA
cggaggccctttcgtcttcaagagaccgggttggcggcg

SEQ ID NO: 81 - DNA, 40 bp, synthetic construct
  source 1..40: mol_type = other DNA
gacgagtcagacaggaggcatcagacagatactcgtcgcg

SEQ ID NO: 82 - DNA, 40 bp, synthetic construct
  source 1..40: mol_type = other DNA
cgcgacgagtatctgtctgatgcctcctgtctgactcgtc

SEQ ID NO: 83 - DNA, 44 bp, synthetic construct
  source 1..44: mol_type = other DNA
atgacgagtcagacaggaggcatggtggtattgtgactggggat

SEQ ID NO: 84 - DNA, 44 bp, synthetic construct
  source 1..44: mol_type = other DNA
atccccagtcacaataccaccatgcctcctgtctgactcgtcat

SEQ ID NO: 85 - DNA, 44 bp, synthetic construct
  source 1..44: mol_type = other DNA
cggcgtccttctcgtagtccgcttttggtggtgaagaggagact

SEQ ID NO: 86 - DNA, 44 bp, synthetic construct
  source 1..44: mol_type = other DNA
agtctcctcttcaccaccaaaagcggactacgagaaggacgccg

SEQ ID NO: 87 - DNA, 30 bp, synthetic construct
  source 1..30: mol_type = other DNA
ccactcgtcaccaacagtgccgtgtgttgc

SEQ ID NO: 88 - DNA, 24 bp, synthetic construct
  source 1..24: mol_type = other DNA
tcgtacgtctataccaacagatgg

SEQ ID NO: 89 - DNA, 24 bp, synthetic construct
  source 1..24: mol_type = other DNA
cgcatacacacacactgccggggg

SEQ ID NO: 90 - DNA, 550 bp, Yarrowia lipolytica
  source 1..550: mol_type = genomic DNA
tccacacgtcgttcttttttccttagccttttttgcagtgcgcgtgtcccaaaccccagctctacacaccagcacaaacaaagttaagctcagggttgtcgttgaggtcgcttactgtagtcagtgctcgtatggttcgttcaattttcgccaaaaatcgttttgcctttgtatcttgggaataacatcaactgtggttcttcaacaggcctaaggaacgaaacaagccggaccaagatcaggttcaaggtgagtactgagaaggaatagaaggcctaaaggcgcaaaccgacaggtggcaacagctccacaccgaccacgaaggccacgaaatcaaggggtcctaaagttagtctttgtggcctcgacggtcagcgaaaacgcgagaccacaacgcgatcagaaccaggacctaaacaacacaggacggggtcacaataggcttgaacagcaagtacaagctgtgatctctctatatttgattctcaaaccacccctgactacttcagcgcctctgtgacacagcccccctatcatccgactaacacag

SEQ ID NO: 91 - DNA, 31 bp, synthetic construct
  source 1..31: mol_type = other DNA
gacaatgcctcgaggaggtttaaaagtaact

SEQ ID NO: 92 - DNA, 41 bp, synthetic construct
  source 1..41: mol_type = other DNA
gcgccgccaacccggtctctctgtgttagtcggatgatagg

SEQ ID NO: 93 - DNA, 41 bp, synthetic construct
  source 1..41: mol_type = other DNA
cctatcatccgactaacacagagagaccgggttggcggcgc

SEQ ID NO: 94 - DNA, 42 bp, synthetic construct
  source 1..42: mol_type = other DNA
gacgagtcagacaggaggcactgcggttagtactgcaaaaag

SEQ ID NO: 95 - DNA, 42 bp, synthetic construct
  source 1..42: mol_type = other DNA
ctttttgcagtactaaccgcagtgcctcctgtctgactcgtc

SEQ ID NO: 96 - DNA, 44 bp, synthetic construct
  source 1..44: mol_type = other DNA
atgcgccgccaacccggtctcttggtggtattgtgactggggat

SEQ ID NO: 97 - DNA, 44 bp, synthetic construct
  source 1..44: mol_type = other DNA
atccccagtcacaataccaccaagagaccgggttggcggcgcat

SEQ ID NO: 98 - DNA, 41 bp, synthetic construct
  source 1..41: mol_type = other DNA
ctttccaatagctgcttgtagctgcggttagtactgcaaaa

SEQ ID NO: 99 - DNA, 41 bp, synthetic construct
  source 1..41: mol_type = other DNA
ttttgcagtactaaccgcagctacaagcagctattggaaag

SEQ ID NO: 100 - DNA, 30 bp, synthetic construct
  source 1..30: mol_type = other DNA
gcttaatgtgattgatctcaaacttgatag

SEQ ID NO: 101 - DNA, 24 bp, synthetic construct
  source 1..24: mol_type = other DNA
gctgtctctgcgagagcacgtcga

SEQ ID NO: 102 - DNA, 24 bp, synthetic construct
  source 1..24: mol_type = other DNA
ggttcgcacaacttctcgggtggc

SEQ ID NO: 103 - protein, 338 aa, Haematococcus pluvialis
MIRAMHNRAPTPRTRVSHPRSHRALAHVSAVATAGQVAEVHSAPAFDFEMYMRDRAEMVNKALDAALPSRYPEVLVDSMRYSVLAGGKRVRPALTLAACDLVGGDMATALPTACAMEMIHTMSLIHDDLPAMDNDDFRRGRPTNHKVYGEDIAILAGDALLSFAFEHIARDTKGVPADAVLKVIMELGRAVGAQGLSAGQAVDIKSEGQEVGLEVLEYIHHHKTAALLEAAVVCGALVGGADTATVEKLRKYALNIGLAFQVIDDILDVTQTTETLGKTAAKDLAVNKTTYPKLLGLEASRKVADDLIREAIAQLDEFEPARKAPMVALAHLIGYRKN